European Patent Application EP 4 714 978 A1, published March 25, 2026. Title: 靶向DLL3的抗体及其应用. Applicant: 星奕昂（上海）生物科技有限公司. The sequence listing filed with the application follows.

SEQUENCE LISTING (74 sequences)

SEQ ID NO: 1 - protein, 5 aa, synthetic construct
  source 1..5: note = Ab.53 VH CDR1
NYAVN

SEQ ID NO: 2 - protein, 17 aa, synthetic construct
  source 1..17: note = Ab.53 VH CDR2
LINTYTENPTYAQDFTG

SEQ ID NO: 3 - protein, 7 aa, synthetic construct
  source 1..7: note = Ab.53 VH CDR3
GMGVFDI

SEQ ID NO: 4 - protein, 16 aa, synthetic construct
  source 1..16: note = Ab.53 VL CDR1
RSSQSLLESNGYNYLD

SEQ ID NO: 5 - protein, 7 aa, synthetic construct
  source 1..7: note = Ab.53 VL CDR2
LGSNRAS

SEQ ID NO: 6 - protein, 9 aa, synthetic construct
  source 1..9: note = Ab.53 VL CDR3
MQALQTPLT

SEQ ID NO: 7 - protein, 5 aa, synthetic construct
  source 1..5: note = Ab.55 VH CDR1
NSYWG

SEQ ID NO: 8 - protein, 16 aa, synthetic construct
  source 1..16: note = Ab.55 VH CDR2
YIYYSGTSSYNPSLES

SEQ ID NO: 9 - protein, 6 aa, synthetic construct
  source 1..6: note = Ab.55 VH CDR3
EGSFDV

SEQ ID NO: 10 - protein, 16 aa, synthetic construct
  source 1..16: note = Ab.55 VL CDR1
RSSQSLLYSDGNTYLI

SEQ ID NO: 11 - protein, 7 aa, synthetic construct
  source 1..7: note = Ab.55 VL CDR2
KLSTRDS

SEQ ID NO: 12 - protein, 9 aa, synthetic construct
  source 1..9: note = Ab.55 VL CDR3
MQVTHWPYT

SEQ ID NO: 13 - protein, 5 aa, synthetic construct
  source 1..5: note = Ab.63 VH CDR1
SYYWS

SEQ ID NO: 14 - protein, 16 aa, synthetic construct
  source 1..16: note = Ab.63 VH CDR2
YIYYSGTTNFNPSLKS

SEQ ID NO: 15 - protein, 10 aa, synthetic construct
  source 1..10: note = Ab.63 VH CDR3
LALTGFHFDY

SEQ ID NO: 16 - protein, 12 aa, synthetic construct
  source 1..12: note = Ab.63 VL CDR1
RASQSVTRGYLA

SEQ ID NO: 17 - protein, 7 aa, synthetic construct
  source 1..7: note = Ab.63 VL CDR2
GASNRAT

SEQ ID NO: 18 - protein, 9 aa, synthetic construct
  source 1..9: note = Ab.63 VL CDR3
QQYGISPLT

SEQ ID NO: 19 - protein, 5 aa, synthetic construct
  source 1..5: note = Ab.67 VH CDR1
GSSMH

SEQ ID NO: 20 - protein, 19 aa, synthetic construct
  source 1..19: note = Ab.67 VH CDR2
RIRNKANNYATSYGASVQG

SEQ ID NO: 21 - protein, 5 aa, synthetic construct
  source 1..5: note = Ab.67 VH CDR3
LSGEF

SEQ ID NO: 22 - protein, 16 aa, synthetic construct
  source 1..16: note = Ab.67 VL CDR1
RSSQSLVYSDGNTYLN

SEQ ID NO: 23 - protein, 7 aa, synthetic construct
  source 1..7: note = Ab.67 VL CDR2
QVSNRDS

SEQ ID NO: 24 - protein, 9 aa, synthetic construct
  source 1..9: note = Ab.67 VL CDR3
MQGTHWPHT

SEQ ID NO: 25 - protein, 5 aa, synthetic construct
  source 1..5: note = Ab.71 VH CDR1
NCGMH

SEQ ID NO: 26 - protein, 17 aa, synthetic construct
  source 1..17: note = Ab.71 VH CDR2
IIWYDGNIKYYGDSVKG

SEQ ID NO: 27 - protein, 10 aa, synthetic construct
  source 1..10: note = Ab.71 VH CDR3
HDYGGNSFDY

SEQ ID NO: 28 - protein, 17 aa, synthetic construct
  source 1..17: note = Ab.71 VL CDR1
KSSQNVLPNSNKKHYLS

SEQ ID NO: 29 - protein, 7 aa, synthetic construct
  source 1..7: note = Ab.71 VL CDR2
LASTRAS

SEQ ID NO: 30 - protein, 11 aa, synthetic construct
  source 1..11: note = Ab.71 VL CDR3
QQYYSSPPEWT

SEQ ID NO: 31 - protein, 5 aa, synthetic construct
  source 1..5: note = Ab.73 VH CDR1
SHYWS

SEQ ID NO: 32 - protein, 16 aa, synthetic construct
  source 1..16: note = Ab.73 VH CDR2
YIYYTGTTNYNPSLKS

SEQ ID NO: 33 - protein, 6 aa, synthetic construct
  source 1..6: note = Ab.73 VH CDR3
EGTFDI

SEQ ID NO: 34 - protein, 16 aa, synthetic construct
  source 1..16: note = Ab.73 VL CDR1
RSSQSLGYSDGDTYLI

SEQ ID NO: 35 - protein, 7 aa, synthetic construct
  source 1..7: note = Ab.73 VL CDR2
KVSNRDS

SEQ ID NO: 36 - protein, 9 aa, synthetic construct
  source 1..9: note = Ab.73 VL CDR3
MQGTHWPYT

SEQ ID NO: 37 - protein, 5 aa, synthetic construct
  source 1..5: note = Ab.76 VH CDR1
DYAMH

SEQ ID NO: 38 - protein, 17 aa, synthetic construct
  source 1..17: note = Ab.76 VH CDR2
VISWNSGSIGYADSVKG

SEQ ID NO: 39 - protein, 11 aa, synthetic construct
  source 1..11: note = Ab.76 VH CDR3
DLEGGVMDFDY

SEQ ID NO: 40 - protein, 11 aa, synthetic construct
  source 1..11: note = Ab.76 VL CDR1
RASQSVSSNLA

SEQ ID NO: 41 - protein, 7 aa, synthetic construct
  source 1..7: note = Ab.76 VL CDR2
GAYTRAT

SEQ ID NO: 42 - protein, 9 aa, synthetic construct
  source 1..9: note = Ab.76 VL CDR3
QQYNNWPFT

SEQ ID NO: 43 - protein, 16 aa, synthetic construct
  source 1..16: note = Ab.79 VH CDR2
YMYYSGTTNYNPSLTN

SEQ ID NO: 44 - protein, 16 aa, synthetic construct
  source 1..16: note = Ab.79 VL CDR1
RSSQSLVYNDGNTYLT

SEQ ID NO: 45 - protein, 7 aa, synthetic construct
  source 1..7: note = Ab.53 VH CDR1
GYAFSNY

SEQ ID NO: 46 - protein, 6 aa, synthetic construct
  source 1..6: note = Ab.53 VH CDR2
NTYTEN

SEQ ID NO: 47 - protein, 7 aa, synthetic construct
  source 1..7: note = Ab.55 VH CDR1
GDSLKNS

SEQ ID NO: 48 - protein, 5 aa, synthetic construct
  source 1..5: note = Ab.55 VH CDR2
YYSGT

SEQ ID NO: 49 - protein, 7 aa, synthetic construct
  source 1..7: note = Ab.63 VH CDR1
GASISSY

SEQ ID NO: 50 - protein, 7 aa, synthetic construct
  source 1..7: note = Ab.67 VH CDR1
GFIFSGS

SEQ ID NO: 51 - protein, 8 aa, synthetic construct
  source 1..8: note = Ab.67 VH CDR2
RNKANNYA

SEQ ID NO: 52 - protein, 7 aa, synthetic construct
  source 1..7: note = Ab.71 VH CDR1
GFTFSNC

SEQ ID NO: 53 - protein, 6 aa, synthetic construct
  source 1..6: note = Ab.71 VH CDR2
WYDGNI

SEQ ID NO: 54 - protein, 7 aa, synthetic construct
  source 1..7: note = Ab.73 VH CDR1
TGSFSSH

SEQ ID NO: 55 - protein, 5 aa, synthetic construct
  source 1..5: note = Ab.73 VH CDR2
YYTGT

SEQ ID NO: 56 - protein, 7 aa, synthetic construct
  source 1..7: note = Ab.76 VH CDR1
GFTFDDY

SEQ ID NO: 57 - protein, 6 aa, synthetic construct
  source 1..6: note = Ab.76 VH CDR2
SWNSGS

SEQ ID NO: 58 - protein, 7 aa, synthetic construct
  source 1..7: note = Ab.79 VH CDR1
GGSFRSY

SEQ ID NO: 59 - protein, 242 aa, synthetic construct
  source 1..242: note = Ab.76 scFv
EIVMTQSPATLSVSPGERATLSCRASQSVSSNLAWYRQKPGQAPRLFIYGAYTRATDIPARFSGSGSGTEFTLTISSLQSEDFAVYYCQQYNNWPFTFGPGTKVDIKGGGGSGGGGSGGGGSEVQMVESGGVLVQPGMSLRLSCAASGFTFDDYAMHWVRQPPGKGLEWVSVISWNSGSIGYADSVKGRFTISRDNAKNSLYLQMNSLRAEDTAFYYCAKDLEGGVMDFDYWGQGTLVTVSS

SEQ ID NO: 60 - protein, 241 aa, synthetic construct
  source 1..241: note = Ab.55 scFv
EVVMTQSPLSLPVTLGQPASVSCRSSQSLLYSDGNTYLIWFQQRPGQSPRRLLYKLSTRDSGVPDRFSGSGSGTDFTLKISRVEAEDVGIYYCMQVTHWPYTFGQGTKLEIKGGGGSGGGGSGGGGSQVQLRESGPGLVKPSETLSLTCTVSGDSLKNSYWGWIRQPPGKGLEWIGYIYYSGTSSYNPSLESRVTFSADTSKNQFSLKLSSVTAADTAVYYCSREGSFDVWGRGTLVTVSS

SEQ ID NO: 61 - protein, 243 aa, synthetic construct
  source 1..243: note = Ab.67 scFv
DVVVTQSPLSLPVTLGQPASISCRSSQSLVYSDGNTYLNWFQQRPGQSPRRLVYQVSNRDSGVPDRFSGSGSGTDFTLKISGMEAEDAGVYYCMQGTHWPHTFGQGTKLEIKGGGGSGGGGSGGGGSEVHLVESGGGLVQPGGSLKLSCAASGFIFSGSSMHWVRQASGKGLEWIGRIRNKANNYATSYGASVQGRFTMSRDDSKNTAYLQMNSLKAEDTAVYYCTYLSGEFWGQGTLVTVSS

SEQ ID NO: 62 - protein, 241 aa, synthetic construct
  source 1..241: note = Ab.73 scFv
DVVMTQSPLSLPVTLGQPASISCRSSQSLGYSDGDTYLIWFLQRPGQSPRRLIYKVSNRDSGVPDRFSGSGSGTDFTLKISRVEAEDVGVYYCMQGTHWPYTFGQGTKLEIKGGGGSGGGGSGGGGSQVQVQESGPGLVKPSETLSLTCTVSTGSFSSHYWSWIRQPPGKSLEYIGYIYYTGTTNYNPSLKSRVTISVDTSKNQFSLNVNSVTAADTAVYYCAREGTFDIWGQGTMVTVSS

SEQ ID NO: 63 - protein, 249 aa, synthetic construct
  source 1..249: note = Ab.71 scFv
DIGMTQSPDSLAVSLGERATINCKSSQNVLPNSNKKHYLSWYQQKPGQPPKLLIYLASTRASGVPDRFSGSGSGTDFTLTISSLQAEDVAVYYCQQYYSSPPEWTFGQGTKVEIKGGGGSGGGGSGGGGSQVQLVESGGGVVQPGRSLRLSCVASGFTFSNCGMHWVRQAPGKGLEWVAIIWYDGNIKYYGDSVKGRFTISRDNSKNTLYLQMNSLRVEDTAVYYCGRHDYGGNSFDYWGQGTLVTVSS

SEQ ID NO: 64 - protein, 243 aa, synthetic construct
  source 1..243: note = Ab.53 scFv
DIVMTQSPLSLSVTPGEPASISCRSSQSLLESNGYNYLDWYLQKPGQSPQLLIYLGSNRASGVPDRFSGSGSGTDFTLKISRVEAEDVGIYYCMQALQTPLTFGGGTKVEIRGGGGSGGGGSGGGGSQVQLVQSGSELKKPGASVKVSCKASGYAFSNYAVNWVRQAPGQGLEWMGLINTYTENPTYAQDFTGRFVFSLDTSVTTAYLQITSLKTEDTAVYYCARGMGVFDIWGQGTMVTVSS

SEQ ID NO: 65 - protein, 241 aa, synthetic construct
  source 1..241: note = Ab.79 scFv
DVVMTQSPLSLPVTLGQPASISCRSSQSLVYNDGNTYLTWFQQWPGQSPRRLIYKVSNRDSGVPDRFSGSGSGTDFTLKISRVEAEDIGVYHCMQGTHWPYTFGQGTKLEIKGGGGSGGGGSGGGGSQVQVQESGPGLVKSSETLSLTCTVSGGSFRSYYWSWIRQPPGKGLDYIGYMYYSGTTNYNPSLTNRVSISVDTSKNQFSLKLNSVTAADTAVYYCAREGTFDIWGQGTVVTVSS

SEQ ID NO: 66 - protein, 241 aa, synthetic construct
  source 1..241: note = Ab.63 scFv
QIVLTQSPGTLSLSPGERATLSCRASQSVTRGYLAWYQQKPGQAPRLLFYGASNRATDIPDRFSGSGSGTDFTLIISRLEPEDFAVYYCQQYGISPLTFGGGTKVEIKGGGGSGGGGSGGGGSQVQLHESGPGLVKPSETLSLTCTVSGASISSYYWSWIRQPPGKGLEWIGYIYYSGTTNFNPSLKSRVTISVDTSKNQFSLRLSSVTTADTAVYYCANLALTGFHFDYWGQGTLVTVSS

SEQ ID NO: 67 - protein, 241 aa, synthetic construct
  source 1..241: note = AMG757 scFv
EIVLTQSPGTLSLSPGERVTLSCRASQRVNNNYLAWYQQRPGQAPRLLIYGASSRATGIPDRFSGSGSGTDFTLTISRLEPEDFAVYYCQQYDRSPLTFGCGTKLEIKGGGGSGGGGSGGGGSQVQLQESGPGLVKPSETLSLTCTVSGGSISSYYWSWIRQPPGKCLEWIGYVYYSGTTNYNPSLKSRVTISVDTSKNQFSLKLSSVTAADTAVYYCASIAVTGFYFDYWGQGTLVTVSS

SEQ ID NO: 68 - protein, 24 aa, synthetic construct
  source 1..24: note = IL-21SP
MRSSPGNMERIVICLMVIFLGTLV

SEQ ID NO: 69 - protein, 21 aa, synthetic construct
  source 1..21: note = CD8alphaSP
MALPVTALLLPLALLLHAARP

SEQ ID NO: 70 - protein, 17 aa, synthetic construct
  source 1..17: note = CSF2SP
MWLQSLLLLGTVACSIS

SEQ ID NO: 71 - protein, 21 aa, synthetic construct
  source 1..21: note = DAP12SP
MGGLEPCSRLLLLPLLLAVSG

SEQ ID NO: 72 - protein, 16 aa, synthetic construct
  source 1..16: note = CD16SP
MWQLLLPTALLLLVSA

SEQ ID NO: 73 - protein, 19 aa, synthetic construct
  source 1..19: note = CD56SP
MLQTKDLIWTLFFLGTAVS

SEQ ID NO: 74 - protein, 20 aa, synthetic construct
  source 1..20: note = IL-8SP
MTSKLAVALLAAFLISAALC